European Patent Specification EP 3 938 784 B1, published April 29, 2026. Title: Biological membrane remodling for novel therapeutic approaches. Applicant: Wöll Steffen Schiller Stefan Geißler Simon Scherließ Regina. The sequence listing filed with the application follows.

SEQUENCE LISTING (4 sequences)

SEQ ID NO: 1 - protein, 186 aa, Homo sapiens
MGHHHHHHSSGLVPRGSGMKETAAAKFERQHMDSPDLGTQAKPQIPKDKSKVAGYIEIPDADIKEPVYPGPATREQLNRGVSFAKENASLDDQNISIAGHTFIDRPNYQFTNLKAAKKGSMVYFKVGNETRKYKMTSIRNVKPTAVEVLDEQKGKDKQLTLITCDDYNEETGVWETRKIFVATEVK

SEQ ID NO: 2 - protein, 132 aa, Homo sapiens
QVQLQESGGGLVQAGGSHNLSCTASGITFSSLAMGWFRQTPGKEREFVANIMRSGSSVFYADSVRGRFTISRDNAKNTAHLQMNSLKPEDTAVYFCAATRGAWPAEYWGQGTQVTVSSGGLPETGGHHHHHH

SEQ ID NO: 3 - protein, 129 aa, Homo sapiens
QVQLQESGGALVQPGGSLRLSCAASGFPVNRYSMRWYRQAPGKEREWVAGMSSAGDRSSYEDSVKGRFTISRDDARNTVYLQMNSLKPEDTAVYYCNVNVGFEYWGQGTQVTVSSGGLPETGGHHHHHH

SEQ ID NO: 4 - protein, 245 aa, Aequorea victoria
MVSKGEELFTGVVPILVELDGDVNGHKFSVSGEGEGDATYGKLTLKFICTTGKLPVPWPTLVTTLTYGVQCFSRYPDHMKQHDFFKSAMPEGYVQERTIFFKDDGNYKTRAEVKFEGDTLVNRIELKGIDFKEDGNILGHKLEYNYNSHNVYIMADKQKNGIKVNFKIRHNIEDGSVQLADHYQQNTPIGDGPVLLPDNHYLSTQSALSKDPNEKRDHMVLLEFVTAAGITLGMDELYKHHHHHH